European Patent Application EP 4 653 467 A1, published November 26, 2025. Title: 一种CAR分子、包含其的细胞或外泌体及它们的应用. Applicant: 武汉昭智生物技术有限公司. Application WO. The sequence listing filed with the application follows.

SEQUENCE LISTING (12 sequences)

SEQ ID NO: 1 - protein, 266 aa, synthetic construct
MDFQVQIFSFLLISASVIMSRMADIQMTQTTSSLSASLGDRVTISCRASQDISKYLNWYQQKPDGTVKLLIYHTSRLHSGVPSRFSGSGSGTDYSLTISNLEQEDIATYFCQQGNTLPYTFGGGTKLEITGSTSGSGKPGSGEGSTKGEVKLQESGPGLVAPSQSLSVTCTVSGVSLPDYGVSWIRQPPRKGLEWLGVIWGSETTYYNSALKSRLTIIKDNSKSQVFLKMNSLQTDDTAIYYCAKHYYYGGSYAMDYWGQGTSVTV

SEQ ID NO: 2 - protein, 535 aa, synthetic construct
MALPVTALLLPLALLLHAAIPDTEVQLVESGGGLVKPGGSLKLSCAASGFAFSIYDMSWVRQTPEKRLEWVAYISSGGGTYYPDTVKGRFTISRDNAKNTLYLQMSSLKSEDTAMYYCARHSGYGTHWGVLFAYWGQGTLVTVSAGGGGSGGGGSGGGGSDIQMTQTTSSLSASLGDRVTISCRASQDISNYLNWYQQKPDGTVKLLIYYTSILHSGVPSRFSGSGSGTDYSLTISNLEQEDFATYFCQQGNTLPWTFGGGTKLEIKATTTPAPRPPTPAPTIASQPLSLRPEACRPAAGGAVHTRGLDFACDFWVLVVVGGVLACYSLLVTVAFIIFWVRSKRSRLLHSDYMNMTPRRPGPTRKHYQPYAPPRDFAAYRSKRGRKKLLYIFKQPFMRPVQTTQEEDGCSCRFPEEEEGGCELRVKFSRSADAPAYQQGQNQLYNELNLGRREEYDVLDKRRGRDPEMGGKPRRKNPQEGLYNELQKDKMAEAYSEIGMKGERRRGKGHDGLYQGLSTATKDTYDALHMQALPPR

SEQ ID NO: 3 - DNA, 798 bp, synthetic construct
  source 1..798: mol_type = other DNA
atggattttcaggtgcagattttcagcttcctgctaatcagtgcctcagtcataatgtctagaatggccgacatccagatgacccagaccacctccagcctgagcgccagcctgggcgaccgggtgaccatcagctgccgggccagccaggacatcagcaagtacctgaactggtatcagcagaagcccgacggcaccgtcaagctgctgatctaccacaccagccggctgcacagcggcgtgcccagccggtttagcggcagcggctccggcaccgactacagcctgaccatctccaacctggaacaggaagatatcgccacctacttttgccagcagggcaacacactgccctacacctttggcggcggaacaaagctggaaatcaccggcagcacctccggcagcggcaagcctggcagcggcgagggcagcaccaagggcgaggtgaagctgcaggaaagcggccctggcctggtggcccccagccagagcctgagcgtgacctgcaccgtgagcggcgtgagcctgcccgactacggcgtgagctggatccggcagccccccaggaagggcctggaatggctgggcgtgatctggggcagcgagaccacctactacaacagcgccctgaagagccggctgaccatcatcaaggacaacagcaagagccaggtgttcctgaagatgaacagcctgcagaccgacgacaccgccatctactactgcgccaagcactactactacggcggcagctacgccatggactactggggccagggcaccagcgtgaccgtg

SEQ ID NO: 4 - DNA, 1608 bp, synthetic construct
  source 1..1608: mol_type = other DNA
atggccttaccagtgaccgccttgctcctgccgctggccttgctgctccacgccgccattcccgacactgaagtccagctcgtggaatctggagggggcctggtgaaacctgggggatctctcaaactgtcttgtgccgcttctggctttgcttttagcatctacgacatgtcctgggtccggcagacacctgaaaaacgcctggagtgggtcgcctacatttctagtgggggcggaacatactaccccgataccgtgaagggacgctttacaatttctagggataacgccaaaaacaccctgtacctccagatgtcatccctgaaatctgaggatactgccatgtactactgtgctaggcattctggctacggaacacattggggagtgctcttcgcttactggggccaggggactctcgtcactgtctctgctggcgggggaggctctggcggaggcggatccggaggcggagggagtgatattcagatgactcagaccacctcttctctgtccgcttctctgggcgatagagtgacaatctcctgtcgggcatcacaggatattagcaattacctgaactggtaccagcagaaacccgatggaaccgtcaaactgctcatctactacacctccatcctccactctggcgtgccatctcgattttctggatctggctctggaaccgactactctctcacaatctccaacctggaacaggaggattttgccacctacttttgtcagcagggcaatactctgccttggacctttgggggcggaaccaaactggaaatcaaggccaccacgacgccagcgccgcgaccaccaacaccggcgcccaccatcgcgtcgcagcccctgtccctgcgcccagaggcgtgccggccagcggcggggggcgcagtgcacacgagggggctggacttcgcctgtgatttttgggtgctggtggtggttggtggagtcctggcttgctatagcttgctagtaacagtggcctttattattttctgggtgaggagtaagaggagcaggctcctgcacagtgactacatgaacatgactccccgccgccccgggcccacccgcaagcattaccagccctatgccccaccacgcgacttcgcagcctatcgctccaaacggggcagaaagaaactcctgtatatattcaaacaaccatttatgagaccagtacaaactactcaagaggaagatggctgtagctgccgatttccagaagaagaagaaggaggatgtgaactgagagtgaagttcagcaggagcgcagacgcccccgcgtaccagcagggccagaaccagctctataacgagctcaatctaggacgaagagaggagtacgatgttttggacaagagacgtggccgggaccctgagatggggggaaagccgagaaggaagaaccctcaggaaggcctgtacaatgaactgcagaaagataagatggcggaggcctacagtgagattgggatgaaaggcgagcgccggaggggcaaggggcacgatggcctttaccagggtctcagtacagccaccaaggacacctacgacgcccttcacatgcaggccctgccccctcgctaa

SEQ ID NO: 5 - DNA, 714 bp, synthetic construct
  source 1..714: mol_type = other DNA
atggcggtggaaggaggaatgaaatgtgtgaagttcttgctctacgtcctcctgctggccttttgcgcctgtgcagtgggactgattgccgtgggtgtcggggcacagcttgtcctgagtcagaccataatccagggggctacccctggctctctgttgccagtggtcatcatcgcagtgggtgtcttcctcttcctggtggcttttgtgggctgctgcggggcctgcaaggagaactattgtcttatgatcacgtttgccatctttctgtctcttatcatgttggtggaggtggccgcagccattgctggctatgtgtttagagataaggtgatgtcagagtttaataacaacttccggcagcagatggagaattacccgaaaaataaccacactgcttcgatcctggacaggatgcaggcagattttaagtgctgtggggctgctaactacacagattgggagaaaatcccttccatgtcgaagaaccgagtccccgactcctgctgcattaatgttactgtgggctgtgggattaatttcaacgagaaggcgatccataaggagggctgtgtggagaagattgggggctggctgaggaaaaatgtgctggtggtagctgcagcagcccttggaattgcttttgtcgaggttttgggaattgtctttgcctgctgcctcgtgaagagtatcagaagtggctacgaggtgatg

SEQ ID NO: 6 - protein, 238 aa, synthetic construct
MAVEGGMKCVKFLLYVLLLAFCACAVGLIAVGVGAQLVLSQTIIQGATPGSLLPVVIIAVGVFLFLVAFVGCCGACKENYCLMITFAIFLSLIMLVEVAAAIAGYVFRDKVMSEFNNNFRQQMENYPKNNHTASILDRMQADFKCCGAANYTDWEKIPSMSKNRVPDSCCINVTVGCGINFNEKAIHKEGCVEKIGGWLRKNVLVVAAAALGIAFVEVLGIVFACCLVKSIRSGYEVM

SEQ ID NO: 7 - DNA, 1665 bp, synthetic construct
  source 1..1665: mol_type = other DNA
atggcagcccgtctgctcctcctgggcatccttctcctgctgctgcccctgcccgtccctgccccgtgccacacagccgcacgctcagagtgcaagcgcagccacaagttcgtgcctggtgcatggctggccggggagggtgtggacgtgaccagcctccgccgctcgggctccttcccagtggacacacaaaggttcctgcggcccgacggcacctgcaccctctgtgaaaatgccctacaggagggcaccctccagcgcctgcctctggcgctcaccaactggcgggcccagggctctggctgccagcgccatgtaaccagggccaaagtcagctccactgaagctgtggcccgggatgcggctcgtagcatccgcaacgactggaaggtcgggctggacgtgactcctaagcccaccagcaatgtgcatgtgtctgtggccggctcacactcacaggcagccaactttgcagcccagaagacccaccaggaccagtacagcttcagcactgacacggtggagtgccgcttctacagtttccatgtggtacacactcccccgctgcaccctgacttcaagagggccctcggggacctgccccaccacttcaacgcctccacccagcccgcctacctcaggcttatctccaactacggcacccacttcatccgggctgtggagctgggtggccgcatatcggccctcactgccctgcgcacctgcgagctggccctggaagggctcacggacaacgaggtggaggactgcctgactgtcgaggcccaggtcaacataggcatccacggcagcatctctgccgaagccaaggcctgtgaggagaagaagaagaagcacaagatgacggcctccttccaccaaacctaccgggagcgccattcggaagtggttggcggccatcacacctccattaacgacctgctgttcgggatccaggccgggcccgagcagtactcagcctgggtaaactcgctgcccggcagccctggcctggtggactacaccctggaacccctgcacgtgctgctggacagccaggacccgcggcgggaggcactgaggagggccctgagtcagtacctgacggacagggctcgctggagggactgcagccggccgtgcccaccagggcggcagaagagcccccgagacccatgccagtgtgtgtgccatggctcagcggtcaccacccaggactgctgccctcggcagaggggcctggcccagctggaggtgaccttcatccaagcatggggcctgtggggggactggttcactgccacggatgcctatgtgaagctcttctttggtggccaggagctgaggacgagcaccgtgtgggacaataacaaccccatctggtcagtgcggctggattttggggatgtgctcctggccacaggggggcccctgaggttgcaggtctgggatcaggactctggcagggacgatgacctccttggcacctgtgatcaggctcccaagtctggttcccatgaggtgagatgcaacctgaatcatggccacctaaaattccgctatcatgccaggtgcttgccccacctgggaggaggcacctgcctggactatgtcccccaaatgcttctgggggagcctccaggaaaccggagtggggccgtgtgg

SEQ ID NO: 8 - protein, 555 aa, synthetic construct
MAARLLLLGILLLLLPLPVPAPCHTAARSECKRSHKFVPGAWLAGEGVDVTSLRRSGSFPVDTQRFLRPDGTCTLCENALQEGTLQRLPLALTNWRAQGSGCQRHVTRAKVSSTEAVARDAARSIRNDWKVGLDVTPKPTSNVHVSVAGSHSQAANFAAQKTHQDQYSFSTDTVECRFYSFHVVHTPPLHPDFKRALGDLPHHFNASTQPAYLRLISNYGTHFIRAVELGGRISALTALRTCELALEGLTDNEVEDCLTVEAQVNIGIHGSISAEAKACEEKKKKHKMTASFHQTYRERHSEVVGGHHTSINDLLFGIQAGPEQYSAWVNSLPGSPGLVDYTLEPLHVLLDSQDPRREALRRALSQYLTDRARWRDCSRPCPPGRQKSPRDPCQCVCHGSAVTTQDCCPRQRGLAQLEVTFIQAWGLWGDWFTATDAYVKLFFGGQELRTSTVWDNNNPIWSVRLDFGDVLLATGGPLRLQVWDQDSGRDDDLLGTCDQAPKSGSHEVRCNLNHGHLKFRYHARCLPHLGGGTCLDYVPQMLLGEPPGNRSGAVW

SEQ ID NO: 9 - DNA, 744 bp, synthetic construct
  source 1..744: mol_type = other DNA
atgcaaccaatcctgcttctgctggccttcctcctgctgcccagggcagatgcaggggagatcatcgggggacatgaggccaagccccactcccgcccctacatggcttatcttatgatctgggatcagaagtctctgaagaggtgcggtggcttcctgatacaagacgacttcgtgctgacagctgctcactgttggggaagctccataaatgtcaccttgggggcccacaatatcaaagaacaggagccgacccagcagtttatccctgtgaaaagacccatcccccatccagcctataatcctaagaacttctccaacgacatcatgctactgcagctggagagaaaggccaagcggaccagagctgtgcagcccctcaggctacctagcaacaaggcccaggtgaagccagggcagacatgcagtgtggccggctgggggcagacggcccccctgggaaaacactcacacacactacaagaggtgaagatgacagtgcaggaagatcgaaagtgcgaatctgacttacgccattattacgacagtaccattgagttgtgcgtgggggacccagagattaaaaagacttcctttaagggggactctggaggccctcttgtgtgtaacaaggtggcccagggcattgtctcctatggacgaaacaatggcatgcctccacgagcctgcaccaaagtctcaagctttgtacactggataaagaaaaccatgaaacgccactaa

SEQ ID NO: 10 - protein, 247 aa, synthetic construct [sequence omitted]

SEQ ID NO: 11 - DNA, 1623 bp, synthetic construct
  source 1..1623: mol_type = other DNA
atgaatactctccctgaacattcatgtgacgtgttgattatcggtagcggcgcagccggactttcactggcgctacgcctggctgaccagcatcaggtcatcgttctaagtaaaggcccggtaacggaaggttcaacattttatgcccagggcggtattgccgccgtgtttgatgaaactgacagcattgactcgcatgtggaagacacattgattgccggggctggtatttgcgatcgccatgcagttgaatttgtcgccagcaatgcacgatcctgtgtgcaatggctaatcgaccagggggtgttgtttgatacccacattcaaccgaatggcgaagaaagttaccatctgacccgtgaaggtggacatagtcaccgtcgtattcttcatgccgccgacgccaccggtagagaagtagaaaccacgctggtgagcaaggcgctgaaccatccgaatattcgcgtgctggagcgcagcaacgcggttgatctgattgtttctgacaaaattggcctgccgggcacgcgacgggttgttggcgcgtgggtatggaaccgtaataaagaaacggtggaaacctgccacgcaaaagcggtggtgctggcaaccggcggtgcgtcgaaggtttatcagtacaccaccaatccggatatttcttctggcgatggcattgctatggcgtggcgcgcaggctgccgggttgccaatctcgaatttaatcagttccaccctaccgcgctatatcacccacaggcacgcaatttcctgttaacagaagcactgcgcggcgaaggcgcttatctcaagcgcccggatggtacgcgttttatgcccgattttgatgagcgcggcgaactggccccgcgcgatattgtcgcccgcgccattgaccatgaaatgaaacgcctcggcgcagattgtatgttccttgatatcagccataagcccgccgattttattcgccagcatttcccgatgatttatgaaaagctgctcgggctggggattgatctcacacaagaaccggtaccgattgtgcctgctgcacattatacctgcggtggtgtaatggttgatgatcatgggcgtacggacgtcgagggcttgtatgccattggcgaggtgagttataccggcttacacggcgctaaccgcatggcctcgaactcattgctggagtgtctggtctatggctggtcggcggcggaagatatcaccagacgtatgccttatgcccacgacatcagtacgttaccgccgtgggatgaaagccgcgttgagaaccctgacgaacgggtagtaattcagcataactggcacgagctacgtctgtttatgtgggattacgttggcattgtgcgcacaacgaagcgcctggaacgcgccctgcggcggataaccatgctccaacaagaaatagacgaatattacgcccatttccgcgtctcaaataatttgctggagctgcgtaatctggtacaggttgccgagttgattgttcgctgtgcaatgatgcgtaaagagagtcgggggttgcatttcacgctggattatccggaactgctcacccattccggtccgtcgatcctttcccccggcaatcattacataaacagataa

SEQ ID NO: 12 - protein, 540 aa, synthetic construct
MNTLPEHSCDVLIIGSGAAGLSLALRLADQHQVIVLSKGPVTEGSTFYAQGGIAAVFDETDSIDSHVEDTLIAGAGICDRHAVEFVASNARSCVQWLIDQGVLFDTHIQPNGEESYHLTREGGHSHRRILHAADATGREVETTLVSKALNHPNIRVLERSNAVDLIVSDKIGLPGTRRVVGAWVWNRNKETVETCHAKAVVLATGGASKVYQYTTNPDISSGDGIAMAWRAGCRVANLEFNQFHPTALYHPQARNFLLTEALRGEGAYLKRPDGTRFMPDFDERGELAPRDIVARAIDHEMKRLGADCMFLDISHKPADFIRQHFPMIYEKLLGLGIDLTQEPVPIVPAAHYTCGGVMVDDHGRTDVEGLYAIGEVSYTGLHGANRMASNSLLECLVYGWSAAEDITRRMPYAHDISTLPPWDESRVENPDERVVIQHNWHELRLFMWDYVGIVRTTKRLERALRRITMLQQEIDEYYAHFRVSNNLLELRNLVQVAELIVRCAMMRKESRGLHFTLDYPELLTHSGPSILSPGNHYINR